European Patent Application EP 4 428 254 A1, published September 11, 2024. Title: Primer set, composition and kit for detection of Vaccinia virus, and method for determination using the same. Applicant: Kolon Industries, Inc. The sequence listing filed with the application follows.

SEQUENCE LISTING (15 sequences)

SEQ ID NO: 1 - DNA, 20 bp, synthetic construct
  source 1..20: mol_type = other DNA
cggacgtgctagggaacaaa

SEQ ID NO: 2 - DNA, 20 bp, synthetic construct
  source 1..20: mol_type = other DNA
ttcgcgagtcaattccctcc

SEQ ID NO: 3 - DNA, 20 bp, synthetic construct
  source 1..20: mol_type = other DNA
ggagggaattgactcgcgaa

SEQ ID NO: 4 - DNA, 20 bp, synthetic construct
  source 1..20: mol_type = other DNA
ggctgctagttgtcgttcga

SEQ ID NO: 5 - DNA, 20 bp, synthetic construct
  source 1..20: mol_type = other DNA
aggctgctagttgtcgttcg

SEQ ID NO: 6 - DNA, 20 bp, synthetic construct
  source 1..20: mol_type = other DNA
acaggctgctagttgtcgtt

SEQ ID NO: 7 - DNA, 20 bp, synthetic construct
  source 1..20: mol_type = other DNA
gcgagtcaattccctcctgt

SEQ ID NO: 8 - DNA, 20 bp, synthetic construct
  source 1..20: mol_type = other DNA
acaggagggaattgactcgc

SEQ ID NO: 9 - DNA, 20 bp, synthetic construct
  source 1..20: mol_type = other DNA
agttgagtgactgcagacgt

SEQ ID NO: 10 - DNA, 20 bp, synthetic construct
  source 1..20: mol_type = other DNA
gatgttccgttaccgttgcg

SEQ ID NO: 11 - DNA, 684 bp, Vaccinia virus IHD-W
  source 1..684: mol_type = genomic DNA
atgaaaccaatgccgaaacagagagagatgcgacgtcttagagatagaatctcagatattgaaagacagttgagtgactgcagacgtaataatgaaagcaatgctgatatggaaagagagatgcaacgtcttagagatagaatcatggatcttgatagacagcttaacgagtgtaaacgcaacggtaacggaacatcttctgaggaggtaaataggctaaagactagaatcaggaatcttaaacgatcgctagagatctgctcaaaggatgaatcagaactctattcagcatataaaactaaactcggacgtgctagggaacaaattagtaacttgcaagaaagtctacgtagagagcgtgaatctgacaaaacagatagttactacaggagggaattgactcgcgaaagaaataaaatcgtagaattggaaaaagaacttaataagtgtttcgatgccaagtacatcgacgaaatcaattccaagaaaacccgtatttctgatctcgaacgacaactagcagcctgtaaatctaatggtggtagcaatggaaacatggaccaatacaaacgggaaattgaatctcttaaacgcgagctcgccgagtgtagacgtggtaacaatggatctcacagtgattgcgcgtactatgacgaagaagcaagagattgtgttaagagctga

SEQ ID NO: 12 - protein, 227 aa, Vaccinia virus IHD-W
MKPMPKQREMRRLRDRISDIERQLSDCRRNNESNADMEREMQRLRDRIMDLDRQLNECKRNGNGTSSEEVNRLKTRIRNLKRSLEICSKDESELYSAYKTKLGRAREQISNLQESLRRERESDKTDSYYRRELTRERNKIVELEKELNKCFDAKYIDEINSKKTRISDLERQLAACKSNGGSNGNMDQYKREIESLKRELAECRRGNNGSHSDCAYYDEEARDCVKS

SEQ ID NO: 13 - DNA, 3642 bp, synthetic construct
  source 1..3642: mol_type = other DNA
gggcgaattgggcccgacgtcgcatgctcccggccgccatggcggccgcgggaattcgattatgaaaccaatgccgaaacagagagagatgcgacgtcttagagatagaatctcagatattgaaagacagttgagtgactgcagacgtaataatgaaagcaatgctgatatggaaagagagatgcaacgtcttagagatagaatcatggatcttgatagacagcttaacgagtgtaaacgcaacggtaacggaacatcttctgaggaggtaaataggctaaagactagaatcaggaatcttaaacgatcgctagagatctgctcaaaggatgaatcagaactctattcagcatataaaactaaactcggacgtgctagggaacaaattagtaacttgcaagaaagtctacgtagagagcgtgaatctgacaaaacagatagttactacaggagggaattgactcgcgaaagaaataaaatcgtagaattggaaaaagaacttaataagtgtttcgatgccaagtacatcgacgaaatcaattccaagaaaacccgtatttctgatctcgaacgacaactagcagcctgtaaatctaatggtggtagcaatggaaacatggaccaatacaaacgggaaattgaatctcttaaacgcgagctcgccgagtgtagacgtggtaacaatgaatcactagtgaattcgcggccgcctgcaggtcgaccatatgggagagctcccaacgcgttggatgcatagcttgagtattctatagtgtcacctaaatagcttggcgtaatcatggtcatagctgtttcctgtgtgaaattgttatccgctcacaattccacacaacatacgagccggaagcataaagtgtaaagcctggggtgcctaatgagtgagctaactcacattaattgcgttgcgctcactgcccgctttccagtcgggaaacctgtcgtgccagctgcattaatgaatcggccaacgcgcggggagaggcggtttgcgtattgggcgctcttccgcttcctcgctcactgactcgctgcgctcggtcgttcggctgcggcgagcggtatcagctcactcaaaggcggtaatacggttatccacagaatcaggggataacgcaggaaagaacatgtgagcaaaaggccagcaaaaggccaggaaccgtaaaaaggccgcgttgctggcgtttttccataggctccgcccccctgacgagcatcacaaaaatcgacgctcaagtcagaggtggcgaaacccgacaggactataaagataccaggcgtttccccctggaagctccctcgtgcgctctcctgttccgaccctgccgcttaccggatacctgtccgcctttctcccttcgggaagcgtggcgctttctcatagctcacgctgtaggtatctcagttcggtgtaggtcgttcgctccaagctgggctgtgtgcacgaaccccccgttcagcccgaccgctgcgccttatccggtaactatcgtcttgagtccaacccggtaagacacgacttatcgccactggcagcagccactggtaacaggattagcagagcgaggtatgtaggcggtgctacagagttcttgaagtggtggcctaactacggctacactagaagaacagtatttggtatctgcgctctgctgaagccagttaccttcggaaaaagagttggtagctcttgatccggcaaacaaaccaccgctggtagcggtggtttttttgtttgcaagcagcagattacgcgcagaaaaaaaggatctcaagaagatcctttgatcttttctacggggtctgacgctcagtggaacgaaaactcacgttaagggattttggtcatgagattatcaaaaaggatcttcacctagatccttttaaattaaaaatgaagttttaaatcaatctaaagtatatatgagtaaacttggtctgacagttaccaatgcttaatcagtgaggcacctatctcagcgatctgtctatttcgttcatccatagttgcctgactccccgtcgtgtagataactacgatacgggagggcttaccatctggccccagtgctgcaatgataccgcgagacccacgctcaccggctccagatttatcagcaataaaccagccagccggaagggccgagcgcagaagtggtcctgcaactttatccgcctccatccagtctattaattgttgccgggaagctagagtaagtagttcgccagttaatagtttgcgcaacgttgttgccattgctacaggcatcgtggtgtcacgctcgtcgtttggtatggcttcattcagctccggttcccaacgatcaaggcgagttacatgatcccccatgttgtgcaaaaaagcggttagctccttcggtcctccgatcgttgtcagaagtaagttggccgcagtgttatcactcatggttatggcagcactgcataattctcttactgtcatgccatccgtaagatgcttttctgtgactggtgagtactcaaccaagtcattctgagaatagtgtatgcggcgaccgagttgctcttgcccggcgtcaatacgggataataccgcgccacatagcagaactttaaaagtgctcatcattggaaaacgttcttcggggcgaaaactctcaaggatcttaccgctgttgagatccagttcgatgtaacccactcgtgcacccaactgatcttcagcatcttttactttcaccagcgtttctgggtgagcaaaaacaggaaggcaaaatgccgcaaaaaagggaataagggcgacacggaaatgttgaatactcatactcttcctttttcaatattattgaagcatttatcagggttattgtctcatgagcggatacatatttgaatgtatttagaaaaataaacaaataggggttccgcgcacatttccccgaaaagtgccacctgatgcggtgtgaaataccgcacagatgcgtaaggagaaaataccgcatcaggaaattgtaagcgttaatattttgttaaaattcgcgttaaatttttgttaaatcagctcattttttaaccaataggccgaaatcggcaaaatcccttataaatcaaaagaatagaccgagatagggttgagtgttgttccagtttggaacaagagtccactattaaagaacgtggactccaacgtcaaagggcgaaaaaccgtctatcagggcgatggcccactacgtgaaccatcaccctaatcaagttttttggggtcgaggtgccgtaaagcactaaatcggaaccctaaagggagcccccgatttagagcttgacggggaaagccggcgaacgtggcgagaaaggaagggaagaaagcgaaaggagcgggcgctagggcgctggcaagtgtagcggtcacgctgcgcgtaaccaccacacccgccgcgcttaatgcgccgctacagggcgcgtccattcgccattcaggctgcgcaactgttgggaagggcgatcggtgcgggcctcttcgctattacgccagctggcgaaagggggatgtgctgcaaggcgattaagttgggtaacgccagggttttcccagtcacgacgttgtaaaacgacggccagtgaattgtaatacgactcactata

SEQ ID NO: 14 - DNA, 23 bp, synthetic construct
  source 1..23: mol_type = other DNA
atgaaaccaatgccgaaacagag

SEQ ID NO: 15 - DNA, 22 bp, synthetic construct
  source 1..22: mol_type = other DNA
cattgttaccacgtctacactc